European Patent Application EP 4 759 323 A2, published June 17, 2026. Title: VASOACTIVE INTESTINAL PEPTIDE (VIP) RECEPTOR ANTAGONISTS. Applicant: Emory University. The sequence listing filed with the application follows.

SEQUENCE LISTING (56 sequences)

SEQ ID NO: 1 - protein, 28 aa, synthetic construct
KPRRPYTDNYTRLRKQMAVKKYLNSILN

SEQ ID NO: 2 - protein, 28 aa, synthetic construct
HSDAVFTDNYTRLRKQMAVKKYLNSILN

SEQ ID NO: 3 - protein, 29 aa, synthetic construct
  VARIANT 7: note = X is T or A
  VARIANT 8: note = X is D, V or S
  VARIANT 10: note = X is Y or C
  VARIANT 12: note = X is R or S
  VARIANT 17: note = X is M or I
  VARIANT 20: note = X is K or N
  VARIANT 21: note = X is K or no amino acid
  VARIANT 25: note = X is N or M
  VARIANT 26: note = X is S or L
KPRRPYXXBXTXLRKQXAVXXKYLXXILN

SEQ ID NO: 4 - protein, 28 aa, synthetic construct
KPRRPYTDNCTRLRKQMAVKKYLNSILN

SEQ ID NO: 5 - protein, 28 aa, synthetic construct
KPRRPYTDNYTRLRKQMAVKKYLNLILN

SEQ ID NO: 6 - protein, 28 aa, synthetic construct
KPRRPYADNYTRLRKQMAVNKYLNLILN

SEQ ID NO: 7 - protein, 28 aa, synthetic construct
KPRRPYAVNYTRLRKQIAVKKYLMSILN

SEQ ID NO: 8 - protein, 28 aa, synthetic construct
KPRRPYAVNYTRLRKQMAVNKYLMSILN

SEQ ID NO: 9 - protein, 29 aa, synthetic construct
KPRRPYADNCTRLRKQIAVNKKYLNSILN

SEQ ID NO: 10 - protein, 28 aa, synthetic construct
KPRRPYTVNYTSLRKQIAVKKYLMLILN

SEQ ID NO: 11 - protein, 28 aa, synthetic construct
KPRRPYTDNCTSLRKQIAVNKYLNLILN

SEQ ID NO: 12 - protein, 28 aa, synthetic construct
KPRRPYAVNCTSLRKQIAVNKYLNSILN

SEQ ID NO: 13 - protein, 28 aa, synthetic construct
KPRRPYAVNCTSLRKQIAVKKYLMSILN

SEQ ID NO: 14 - protein, 29 aa, synthetic construct
KKPRRPYTVNCTSLRKQIAVKKYLMLILN

SEQ ID NO: 15 - protein, 28 aa, synthetic construct
KPRRPYTSDYTRLRKQMAVKKYLNSILN

SEQ ID NO: 16 - protein, 28 aa, synthetic construct
KPRRPYTSDYTRLRKQMAVKKYLNLILN

SEQ ID NO: 17 - protein, 28 aa, synthetic construct
HSDAVFINTKLDKLNTRLVSAQNYMKYR

SEQ ID NO: 18 - protein, 28 aa, synthetic construct
KPRRPYINTKLDKLNTRLVSAQNYMKYR

SEQ ID NO: 19 - protein, 136 aa, synthetic construct
MLLKLKEKASLTLAVGTLPFPSQFNFVPPGRMCRVAGWGRTGVLKPGSDTLQEVKLRLMDPQACSHFRDFDHNLQLCVGNPRKTKSAFKGDSGGPLLCAGVAQGIVSYGRSDAKPPAVFTRISHYRPWINQILQAN

SEQ ID NO: 20 - protein, 697 aa, synthetic construct
DGICKSSDCIKSAARLIQNMDATTEPCTDFFKYACGGWLKRNVIPETSSRYGNFDILRDELEVVLKDVLQEPKTEDIVAVQKAKALYRSCINESAIDSRGGEPLLKLLPDIYGWPVATENWEQKYGASWTAEKAIAQLNSKYGKKVLINLFVGTDDKNSVNHVIHIDQPRLGLPSRDYYECTGIYKEACTAYVDFMISVARLIRQEERLPIDENQLALEMNKVMELEKEIANATAKPEDRNDPMLLYNKMTLAQIQNNFSLEINGKPFSWLNFTNEIMSTVNISITNEEDVVVYAPEYLTKLKPILTKYSARDLQNLMSWRFIMDLVSSLSRTYKESRNAFRKALYGTTSETATWRRCANYVNGNMENAVGRLYVEAAFAGESKHVVEDLIAQIREVFIQTLDDLTWMDAETKKRAEEKALAIKERIGYPDDIVSNDNKLNNEYLELNYKEDEYFENIIQNLKFSQSKQLKKLREKVDKDEWISGAAVVNAFYSSGRNQIVFPAGILQPPFFSAQQSNSLNYGGIGMVIGHEITHGFDDNGRNFNKDGDLVDWWTQQSASNFKEQSQCMVYQYGNFSWDLAGGQHLNGINTLGENIADNGGLGQAYRAYQNYIKKNGEEKLLPGLDLNHKQLFFLNFAQVWCGTYRPEYAVNSIKTDVESPGNFRIIGTLQNSAEFSEAFHCRKNSYMNPEKKCRVW

SEQ ID NO: 21 - protein, 28 aa, synthetic construct
  VARIANT 7: note = X is T or A
  VARIANT 8: note = X is D, V or S
  VARIANT 10: note = X is Y or C
  VARIANT 20: note = X is K or N
  VARIANT 25: note = X is S or L
  VARIANT 12: note = X is R or S
  VARIANT 17: note = X is M or I
  VARIANT 24: note = X is N orM
KPRRPYXXBXTXLRKQXAVXKYLXXILN

SEQ ID NO: 22 - protein, 6 aa, synthetic construct
GGGGSC

SEQ ID NO: 23 - protein, 15 aa, synthetic construct
CASSLEGTGGYEQYF

SEQ ID NO: 24 - protein, 13 aa, synthetic construct
CASSLRDNQAPLF

SEQ ID NO: 25 - protein, 17 aa, synthetic construct
CASSQDEAGGFAETLYF

SEQ ID NO: 26 - protein, 14 aa, synthetic construct
CASSDTGGQDTQYF

SEQ ID NO: 27 - protein, 12 aa, synthetic construct
CASSDAGYEQYF

SEQ ID NO: 28 - protein, 12 aa, synthetic construct
CASSDGGHEQYF

SEQ ID NO: 29 - protein, 15 aa, synthetic construct
CASSLEGTGGYEQYF

SEQ ID NO: 30 - protein, 12 aa, synthetic construct
CASSDAGYEQYF

SEQ ID NO: 31 - protein, 12 aa, synthetic construct
CASSPDSYEQYF

SEQ ID NO: 32 - protein, 14 aa, synthetic construct
CASSGQGNYAEQFF

SEQ ID NO: 33 - protein, 13 aa, synthetic construct
CASSQDRQDEQYF

SEQ ID NO: 34 - protein, 12 aa, synthetic construct
CASSEAGYEQYF

SEQ ID NO: 35 - protein, 12 aa, synthetic construct
CASSPDSYEQYF

SEQ ID NO: 36 - protein, 15 aa, synthetic construct
CASSLEGTGGYEQYF

SEQ ID NO: 37 - protein, 14 aa, synthetic construct
CASSLRGGSYEQYF

SEQ ID NO: 38 - protein, 15 aa, synthetic construct
CTCSAEGTPNSDYTF

SEQ ID NO: 39 - protein, 12 aa, synthetic construct
CASRDSAETLYF

SEQ ID NO: 40 - protein, 13 aa, synthetic construct
CASSLRDNQAPLF

SEQ ID NO: 41 - protein, 14 aa, synthetic construct
CASSGQGNYAEQFF

SEQ ID NO: 42 - protein, 14 aa, synthetic construct
CASSPQGNYAEQFF

SEQ ID NO: 43 - protein, 12 aa, synthetic construct
CASSDAGYEQYF

SEQ ID NO: 44 - protein, 15 aa, synthetic construct
CASSLEGTGGYEQYF

SEQ ID NO: 45 - protein, 14 aa, synthetic construct
CASSDWGSSYEQYF

SEQ ID NO: 46 - protein, 12 aa, synthetic construct
CASSWGQDTQYF

SEQ ID NO: 47 - protein, 14 aa, synthetic construct
CASSLEGSAETLYF

SEQ ID NO: 48 - protein, 12 aa, synthetic construct
CASSDAAETLYF

SEQ ID NO: 49 - protein, 13 aa, synthetic construct
CASSPRNTGQLYF

SEQ ID NO: 50 - protein, 12 aa, synthetic construct
CASRDSAETLYF

SEQ ID NO: 51 - protein, 17 aa, synthetic construct
CASSQDEAGGFAETLYF

SEQ ID NO: 52 - protein, 13 aa, synthetic construct
CASSLRDNQAPLF

SEQ ID NO: 53 - protein, 11 aa, synthetic construct
CASSLEYEQYF

SEQ ID NO: 54 - protein, 12 aa, synthetic construct
CASSPDSYEQYF

SEQ ID NO: 55 - RNA, 100 nt, Mus musculus
  source 1..100: mol_type = mRNA
ggtgagcagcatccatccacaatgtcgctttcatctagaaatacaagaagaagagacaaaatgtgcagagctgctaagcagccaaaggagaatcagagag

SEQ ID NO: 56 - RNA, 101 nt, Mus musculus
  source 1..101: mol_type = mRNA
ggtgagcagcatccatccacaatgtcgctttcatctagaaatacaagaagaagagacaaaatgtgcagagctgctaagcagccaaacggagaatcagagag